European Patent Specification EP 3 452 407 B1, published April 3, 2024. Title: METHODS AND USES FOR REMOTELY TRIGGERED PROTEASE ACTIVITY MEASUREMENTS. Applicant: Massachusetts Institute of Technology. Application Not Yet Assigned. The sequence listing filed with the application follows.

SEQUENCE LISTING (15 sequences)

SEQ ID NO: 1 - protein, 14 aa, Artificial Sequence [sequence omitted]

SEQ ID NO: 2 - protein, 7 aa, Artificial Sequence
  Synthetic polypeptide
  MISC_FEATURE (3)..(4): Modified by a scissile bond
PLGLEEA

SEQ ID NO: 3 - protein, 11 aa, Artificial Sequence
  Synthetic polypeptide
  MISC_FEATURE (1)..(1): Modifed by FAM
  MOD_RES (1)..(1): D stereoisomer of Ser
  MOD_RES (2)..(2): D stereoisomer of Lys
SKPLGLEEAGC

SEQ ID NO: 4 - protein, 9 aa, Artificial Sequence
  Synthetic polypeptide
  MISC_FEATURE (1)..(1): Modified by Biotin-PEG(5 kDa)-(KFAM)
PLGLEEAGC

SEQ ID NO: 5 - protein, 23 aa, Artificial Sequence
  Synthetic polypeptide
  MOD_RES (1)..(1): D stereoisomer of Glu
  MOD_RES (3)..(3): D stereoisomer of Val
  MOD_RES (4)..(4): D stereoisomer of Asn
  MOD_RES (5)..(5): D stereoisomer of Asp
  MOD_RES (6)..(6): D stereoisomer of Asn
  MOD_RES (7)..(7): D stereoisomer of Glu
  MOD_RES (8)..(8): D stereoisomer of Glu
  MOD_RES (10)..(10): D stereoisomer of Phe
  MOD_RES (11)..(11): D stereoisomer of Phe
  MOD_RES (12)..(12): D stereoisomer of Ser
  MOD_RES (13)..(13): D stereoisomer of Ala
  MOD_RES (14)..(14): D stereoisomer of Arg
  MOD_RES (16)..(16): D stereoisomer of Ser
EGVNDNEEGFFSARKSRLVGEGC

SEQ ID NO: 6 - protein, 23 aa, Artificial Sequence
  Synthetic polypeptide
  MISC_FEATURE (1)..(1): Modified by Biotin
  MISC_FEATURE (9)..(10): Modified by Cy7
  MOD_RES (10)..(10): D stereoisomer of Glu
  MOD_RES (12)..(12): D stereoisomer of Val
  MOD_RES (13)..(13): D stereoisomer of Asn
  MOD_RES (14)..(14): D stereoisomer of Asp
  MOD_RES (15)..(15): D stereoisomer of Asn
  MOD_RES (16)..(16): D stereoisomer of Glu
  MOD_RES (17)..(17): D stereoisomer of Glu
  MOD_RES (19)..(19): D stereoisomer of Phe
  MOD_RES (20)..(20): D stereoisomer of Phe
  MOD_RES (21)..(21): D stereoisomer of Ser
  MOD_RES (22)..(22): D stereoisomer of Ala
  MOD_RES (23)..(23): D stereoisomer of Arg
  MISC_FEATURE (23)..(23): Modified by NH2
CGPVGLIGKEGVNDNEEGFFSAR

SEQ ID NO: 7 - protein, 25 aa, Artificial Sequence
  Synthetic polypeptide
  MISC_FEATURE (1)..(1): Modified by Biotin
  MISC_FEATURE (11)..(12): Modified by Cy7
  MOD_RES (12)..(12): D stereoisomer of Glu
  MOD_RES (14)..(14): D stereoisomer of Val
  MOD_RES (15)..(15): D stereoisomer of Asn
  MOD_RES (16)..(16): D stereoisomer of Asp
  MOD_RES (17)..(17): D stereoisomer of Asn
  MOD_RES (18)..(18): D stereoisomer of Glu
  MOD_RES (19)..(19): D stereoisomer of Glu
  MOD_RES (21)..(21): D stereoisomer of Phe
  MOD_RES (22)..(22): D stereoisomer of Phe
  MOD_RES (23)..(23): D stereoisomer of Ser
  MOD_RES (24)..(24): D stereoisomer of Ala
  MOD_RES (25)..(25): D stereoisomer of Arg
  MISC_FEATURE (25)..(25): Modified by NH2
CGPVPLSLVMKEGVNDNEEGFFSAR

SEQ ID NO: 8 - protein, 24 aa, Artificial Sequence
  Synthetic polypeptide
  MISC_FEATURE (1)..(1): Modified by Biotin
  MISC_FEATURE (10)..(11): Modified by Cy7
  MOD_RES (11)..(11): D stereoisomer of Glu
  MOD_RES (13)..(13): D stereoisomer of Val
  MOD_RES (14)..(14): D stereoisomer of Asn
  MOD_RES (15)..(15): D stereoisomer of Asp
  MOD_RES (16)..(16): D stereoisomer of Asn
  MOD_RES (17)..(17): D stereoisomer of Glu
  MOD_RES (18)..(18): D stereoisomer of Glu
  MOD_RES (20)..(20): D stereoisomer of Phe
  MOD_RES (21)..(21): D stereoisomer of Phe
  MOD_RES (22)..(22): D stereoisomer of Ser
  MOD_RES (23)..(23): D stereoisomer of Ala
  MOD_RES (24)..(24): D stereoisomer of Arg
  MISC_FEATURE (24)..(24): Modified by NH2
CGPLGVRGKKEGVNDNEEGFFSAR

SEQ ID NO: 9 - protein, 9 aa, Artificial Sequence
  Synthetic polypeptide
  MISC_FEATURE (1)..(1): Modified by a Reporter
  MISC_FEATURE (3)..(4): Modified by a scissile bond
  MISC_FEATURE (5)..(6): Modified by DMNPE
  MISC_FEATURE (9)..(9): Modified by NP
PLGLEEAGC

SEQ ID NO: 10 - protein, 6 aa, Artificial Sequence
  Synthetic polypeptide
  MISC_FEATURE (6)..(6): Modified by NP
LEEAGC

SEQ ID NO: 11 - protein, 5 aa, Artificial Sequence
  Synthetic polypeptide
  MISC_FEATURE (1)..(1): Modified by FAM
  MOD_RES (1)..(1): D stereoisomer of Ser
  MOD_RES (2)..(2): D stereoisomer of Lys
SKPLG

SEQ ID NO: 12 - protein, 11 aa, Artificial Sequence
  Synthetic polypeptide
  MISC_FEATURE (1)..(1): Modified by 5-carboxy-fluorescein
  MOD_RES (1)..(1): D stereoisomer of Ser
  MOD_RES (2)..(2): D stereoisomer of Lys
  MISC_FEATURE (11)..(11): Modified by an Iron oxide nanoparticle
SKPLGLEEAGC

SEQ ID NO: 13 - protein, 9 aa, Artificial Sequence
  Synthetic polypeptide
  MISC_FEATURE (1)..(1): Modified by Biotin-PEG and Lys-5-carboxy-fluorescein
  MISC_FEATURE (9)..(9): Modified by NP
PLGLEEAGC

SEQ ID NO: 14 - protein, 11 aa, Artificial Sequence
  Synthetic polypeptide
  MISC_FEATURE (1)..(1): Modified by FAM
  MOD_RES (1)..(1): D stereoisomer of Ser
  MOD_RES (2)..(2): D stereoisomer of Lys
  MOD_RES (3)..(3): D stereoisomer of Pro
  MOD_RES (4)..(4): D stereoisomer of Leu
  MOD_RES (6)..(6): D stereoisomer of Leu
  MOD_RES (7)..(7): D stereoisomer of Glu
  MOD_RES (8)..(8): D stereoisomer of Glu
  MOD_RES (9)..(9): D stereoisomer of Ala
SKPLGLEEAGC

SEQ ID NO: 15 - protein, 7 aa, Artificial Sequence
  Synthetic polypeptide
RLVGEGC